European Patent Application EP 4 807 008 A1, published September 16, 2026. Title: Microorganism for producing glutamate family amino acids and a method for producing glutamate family amino acids using the same. Applicant: CJ CheilJedang Corporation. Application KR. The sequence listing filed with the application follows.

SEQUENCE LISTING (41 sequences)

SEQ ID NO: 1 - protein, 397 aa, Thermotoga maritima
MFTPRGFKFAGVHCKIKRKRKDLGIIFSEVPCVAAGVFTTNVVKAAPVIYDMEILKKNPNGIKAVVVNSGVANACTGEQGMINARRMAEKTAEELGVPVESVLVSSTGVIGVQLPMDKVENGIEEAARVLSNDPLPFAEAIMTTDTKVKMHSTKVMIDGKEITVLGIAKGSGMIHPNMATMLSFITTDAKISEEALKKLLKLSVDDSYNMIDVDGDTSTNDMVIVLANGLAGNTTIQPETDGFWKLYEAVHEVNQVLAEKIVEDGEGATKVMEVHVINAPDIKSARLIARSIVSSNLVKTAIYGEDANWGRVIAAAGYSGATFDPEKLDLFFESEAGRIKVAENGQGVSFDEEEAKKILSEKKIRIILDMKQGKETAKAWGCDLTEKYVEINGRYRT

SEQ ID NO: 2 - DNA, 1194 bp, Thermotoga maritima
  source 1..1194: mol_type = genomic DNA
atgttcactcccaggggtttcaagttcgcaggagtacactgcaagataaagagaaaaagaaaagacctaggaatcattttctctgaagttccgtgcgttgccgcgggagtcttcaccaccaacgttgtcaaagcagcaccggtgatttacgacatggagatcctgaaaaagaatccaaacggtatcaaagcggtcgttgtgaacagcggtgtggccaacgcatgtaccggtgaacagggaatgatcaacgcaaggaggatggcagaaaaaacggctgaagagctcggtgttcccgttgaaagtgtcctcgtttcctccacaggggtaataggggttcagcttcccatggataaggtggaaaacggcatagaagaagcggcgagggtgctttcaaacgatcctcttccgtttgccgaggcgatcatgacaaccgacacaaaggtgaagatgcacagcaccaaggtgatgatcgatggaaaagaaatcaccgttctgggaatcgccaagggatccggcatgatccaccccaacatggcaaccatgctctcgttcataacgacagacgcaaaaatttctgaagaagccctgaaaaaactcttaaagctctcagtcgatgattcctacaacatgatagacgtcgatggagacacgagcacgaacgacatggtgatcgttctcgcaaacggtcttgcgggcaacacaacgatccagcccgaaacggatggtttctggaaactctacgaagccgttcacgaggtgaatcaggttctcgcggagaagatagtggaagacggtgagggagcaacgaaagtcatggaagtccatgtaatcaacgcccccgatataaagtcagcgagactgatcgccagatcgatcgtttcctcaaaccttgtgaagacagccatatatggggaggacgcgaactggggaagggtcatcgccgcggcggggtactccggtgcaacctttgatcctgagaaactcgacctgttcttcgaaagcgaggcgggaaggataaaggtggcggaaaacgggcagggagtatctttcgacgaggaagaagcgaagaagattctcagcgaaaagaagataagaataatcctcgacatgaaacagggaaaagagaccgcaaaagcgtggggatgtgatctcacggagaagtacgttgagataaacgggaggtacagaacatga

SEQ ID NO: 3 - DNA, 1194 bp, synthetic construct
  source 1..1194: mol_type = other DNA
atgttcaccccacgcggcttcaagttcgcaggcgtgcactgcaagatcaagcgcaagcgcaaggatctgggcatcatcttctccgaagtgccatgcgttgcagcaggtgtctttaccaccaacgtggtgaaggctgcaccagtgatctacgatatggagatcctcaagaagaacccaaacggcatcaaggctgtcgtggtgaactccggcgtggctaacgcttgcaccggcgaacagggtatgattaacgctcgccgtatggctgaaaagaccgcagaggaactgggtgtcccagtcgaatccgtgctggtgtcctccaccggtgtgattggcgttcagctgccaatggacaaggttgaaaacggcatcgaggaagctgcacgcgtcctgtccaacgacccactgccattcgcagaggcaatcatgaccaccgataccaaggtcaagatgcactctaccaaggtcatgatcgacggcaaggaaatcaccgtgttgggtatcgcaaagggttccggtatgatccacccaaacatggctaccatgctgtccttcatcaccaccgatgctaagatctccgaggaagcactgaaaaagctgctgaaactgtccgtcgatgattcctacaacatgatcgacgtggacggcgatacctccaccaacgatatggtgatcgtgctggctaacggcctggctggcaacaccaccatccagccagaaaccgatggtttctggaagctgtacgaggccgtccacgaagtcaaccaggtgctggctgaaaagatcgttgaagatggcgagggtgcaaccaaggtgatggaagtccacgttatcaacgcacccgatatcaagtccgcacgcctcatcgcacgctccattgtctcctccaacctggttaagaccgctatctacggcgaagatgcaaactggggccgcgtgattgctgctgcaggctactccggcgcaaccttcgatcctgagaagctggatctcttcttcgagtccgaggctggccgcatcaaggtcgctgaaaacggccagggtgtgtctttcgatgaggaagaggcaaagaagatcctgtccgagaagaagatccgcatcatcctggatatgaagcagggcaaggaaaccgcaaaggcttggggttgtgatctgaccgaaaagtacgtcgaaatcaacggtcgctatcgcacctaa

SEQ ID NO: 4 - protein, 397 aa, Thermotoga neapolitana
MFVPRGFSYAGVHCRIKRKRKDLGIIFSEVPCTAAGVFTTNVVKAAPVIYDMEILGKNPSGIRAITVNSGVANACTGEQGMINARRMAEKTAKELNIPVESVLVSSTGVIGVQLPMEKVESGIEEAVKNLSKDPVPFAEAIMTTDTKIKIHSKKVTIEGKEITVLGIAKGSGMIHPNMATMLSFITTDANVSEDALKKLLKISVDDSYNMIDVDGDTSTNDMVIILANGLAGNAPIQEETDGFWKLYEAVHEVNQVLAEKIVEDGEGATKVIEVEVRNAPDRNSARLIARAIVSSNLVKTAIYGEDANWGRVIAAAGYSGAQFDPDRLDLFFESAAGRIKVAENGQGVDFDEDTAKKILSEKKVKIILDMKQGKELARAWGCDLTEKYVEINGRYRT

SEQ ID NO: 5 - DNA, 1194 bp, Thermotoga neapolitana
  source 1..1194: mol_type = genomic DNA
atgttcgttccgaggggattcagctacgcgggagtacactgcagaataaagagaaaaaggaaagacctcggtatcatcttctctgaagtgccctgcaccgccgccggggttttcaccacgaacgttgtgaaggctgcacccgtgatctacgacatggagattctggggaaaaatccttctggaatcagagcgattaccgtgaacagcggtgtagcgaacgcctgcacgggagaacagggaatgatcaacgcaagaaggatggcggagaaaacggcaaaagaactgaacatccccgttgaaagcgtccttgtgtcttcaacaggagtgataggtgttcaacttccaatggaaaaagtggagtcggggattgaagaggcggtgaagaacctctcgaaagaccctgttccctttgcagaggccatcatgacaacggacacgaagataaagatccacagcaaaaaagtgacgatagaagggaaagagatcaccgtccttggaatagcaaagggctccggtatgatacatcccaacatggcgacgatgctctctttcataacgaccgatgcgaatgtttctgaggatgctctgaaaaaacttctgaagatctctgtcgacgattcctacaacatgatcgatgtcgacggtgatacaagcacaaacgacatggtgatcatactcgcaaatggacttgcaggaaacgcacccattcaggaggaaaccgatggtttctggaagctttatgaggccgtacacgaagtcaaccaggtccttgcggaaaaaattgtggaggacggagagggtgccacaaaggtgatagaagtggaagtgagaaatgctccggacagaaactctgctcgtttgattgcacgggcgatcgtctcttcgaatcttgtgaagacagccatctacggtgaagatgcaaactggggaagggtgatagcagccgcggggtactccggtgcacagttcgatccggacagactcgaccttttcttcgaaagcgcagccggtagaataaaggtggcagagaacggccagggagtggattttgacgaagatacagcaaagaagatactgagcgaaaagaaggtgaaaatcatcctcgatatgaagcagggaaaagaacttgcaagagcctggggatgtgatctgactgaaaaatacgtggaaataaacgggaggtacaggacatga

SEQ ID NO: 6 - DNA, 1194 bp, synthetic construct
  source 1..1194: mol_type = other DNA
atgttcgtccctaggggcttctcatacgctggcgtgcactgccgtatcaagcgcaagcgcaaggacctaggtatcatcttcagcgaggtgccatgcaccgctgctggtgttttcaccaccaacgtcgtgaaggctgcaccagtgatctacgatatggaaatcctgggcaagaacccatctggcatccgcgctatcaccgtgaactccggcgttgcaaacgcatgcaccggcgaacagggcatgatcaacgctcgccgcatggctgaaaagaccgcaaaggaactgaacatcccagtggaatccgtgctggtgagctccaccggtgttatcggcgtccagctgccaatggaaaaggtggaatccggcatcgaagaagcagtcaagaacctgtccaaggatccagttccattcgctgaagcaatcatgaccaccgataccaagatcaagatccactctaagaaggtgaccatcgaaggtaaggaaatcaccgtcctcggcatcgctaagggctccggcatgatccacccaaacatggctaccatgctgtccttcatcaccaccgatgcaaacgtgtccgaagatgctctgaagaagctcctgaagatctccgtcgatgattcctacaacatgatcgatgtggatggtgatacctccactaacgacatggtgatcatcctggcaaacggcctggctggtaacgcaccaatccaggaagaaaccgacggcttctggaagctgtacgaagcagtccacgaggtgaaccaggttctggcagaaaagatcgtggaagatggcgaaggcgctaccaaggtgatcgaagttgaggtccgtaacgcaccagatcgcaactccgctcgcctgatcgcacgcgcaatcgtttcctccaacctggttaagaccgcaatctacggcgaggacgcaaactggggccgcgttatcgccgcagccggctactctggcgcacagttcgatccagatcgcctcgacctgttcttcgaatccgctgcaggccgcatcaaggtggcagaaaacggccagggcgtggatttcgatgaagataccgctaagaagatcctgtctgaaaagaaggtgaagatcatcctggatatgaagcagggcaaggaactggcacgcgcttggggttgcgatctgaccgaaaagtacgttgagatcaacggccgctaccgcacctaa

SEQ ID NO: 7 - protein, 388 aa, Corynebacterium glutamicum
MAKKGITAPKGFVASATTAGIKASGNPDMALVVNQGPEFSAAAVFTRNRVFAAPVKVSRENVADGQIRAVLYNAGNANACNGLQGEKDARESVSHLAQNLGLEDSDIGVCSTGLIGELLPMDKLNTGIDQLTAEGALGDNGAAAAKAIMTTDTVDKETVVFADGWTVGGMGKGVGMMAPSLATMLVCLTTDASVTQEMAQIALANATAVTFDTLDIDGSTSTNDTVFLLASGASGITPTQDELNDAVYAACSDIAAKLQADAEGVTKRVAVTVVGTTNNEQAINAARTVARDNLFKCAMFGSDPNWGRVLAAVGMADADMEPEKISVFFNDQAVCLDSTGAPGAREVDLSGADIDVRIDLGTSGEGQATVRTTDLSFSYVEINSAYSS

SEQ ID NO: 8 - DNA, 1167 bp, Corynebacterium glutamicum
  source 1..1167: mol_type = genomic DNA
atggccaaaaaaggcattaccgcgccgaaaggcttcgttgcttctgcaacgaccgcgggtattaaagcttctggcaatcctgacatggcgttggtggttaaccagggtccagagttttccgcagcggccgtgtttacacgcaaccgagttttcgcagcgcctgtgaaggtgagccgggagaacgttgctgatggccagatcagggctgttttgtacaacgctggtaatgctaatgcgtgtaatggtctgcagggtgagaaggatgctcgtgagtctgtttctcatctagctcaaaatttgggcttggaggattccgatattggtgtgtgttccactggtcttattggtgagttgcttccgatggataagctcaatacaggtattgatcagctgaccgctgagggcgctttgggtgacaatggtgcagctgctgccaaggcgatcatgaccactgacacggtggataaggaaaccgtcgtgtttgctgatggttggactgtcggcggaatgggcaagggcgtgggcatgatggcgccgtctcttgccaccatgctggtctgcttgaccactgatgcatccgttactcaggaaatggctcagattgcgctggctaatgctacggccgttacgtttgacaccctggatattgatggatcaacctccaccaatgacaccgtgttcctgctggcatctggcgctagcggaatcaccccaactcaggatgaactcaacgatgcggtgtacgcagcttgttctgatatcgcagcgaagcttcaggctgatgcagagggggtgaccaagcgcgttgctgtgacagtggtgggaaccaccaacaacgagcaggcgatcaatgcggctcgcacggttgctcgtgacaatttgttcaagtgcgcaatgtttggatctgatccaaactggggtcgcgtgttggctgcagtcggcatggctgatgctgatatggaaccagagaagatttctgtgttcttcaatgatcaagcagtatgccttgattccactggcgctcctggtgctcgtgaggtggatctttccggcgctgacattgatgtccgaattgatttgggcaccagtggggaaggccaggcaacagttcgaaccactgacctgagcttctcctacgtggagatcaactccgcgtacagctcttaa

SEQ ID NO: 9 - DNA, 34 bp, synthetic construct
  source 1..34: mol_type = other DNA
caaattcgaaaccgataatgttcgtccctagggg

SEQ ID NO: 10 - DNA, 34 bp, synthetic construct
  source 1..34: mol_type = other DNA
gtggcggccgctctagattaggtgcggtagcggc

SEQ ID NO: 11 - DNA, 34 bp, synthetic construct
  source 1..34: mol_type = other DNA
caaattcgaaaccgataatgttcaccccacgcgg

SEQ ID NO: 12 - DNA, 34 bp, synthetic construct
  source 1..34: mol_type = other DNA
gtggcggccgctctagattaggtgcgatagcgac

SEQ ID NO: 13 - DNA, 34 bp, synthetic construct
  source 1..34: mol_type = other DNA
caaattcgaaaccgataatggccaaaaaaggcat

SEQ ID NO: 14 - DNA, 34 bp, synthetic construct
  source 1..34: mol_type = other DNA
gtggcggccgctctagattaagagctgtacgcgg

SEQ ID NO: 15 - DNA, 34 bp, synthetic construct
  source 1..34: mol_type = other DNA
tgcagcccgggggatcccagccgaagttttaggt

SEQ ID NO: 16 - DNA, 34 bp, synthetic construct
  source 1..34: mol_type = other DNA
tatcggtttcgaatttgggtcagatgtagtcata

SEQ ID NO: 17 - DNA, 36 bp, synthetic construct
  source 1..36: mol_type = other DNA
cggtacccggggatccctcgtgcggaattcgtggag

SEQ ID NO: 18 - DNA, 20 bp, synthetic construct
  source 1..20: mol_type = other DNA
atccagcagcaattcagaca

SEQ ID NO: 19 - DNA, 37 bp, synthetic construct
  source 1..37: mol_type = other DNA
ctgaattgctgctggattaaggcatcgatatcaccca

SEQ ID NO: 20 - DNA, 36 bp, synthetic construct
  source 1..36: mol_type = other DNA
atgcctgcaggtcgacccttcattttaagttccttg

SEQ ID NO: 21 - DNA, 35 bp, synthetic construct
  source 1..35: mol_type = other DNA
cggtacccggggatcctgaccccaggcaagcacgg

SEQ ID NO: 22 - DNA, 27 bp, synthetic construct
  source 1..27: mol_type = other DNA
gaagcgagtacgagtttaagtcttatc

SEQ ID NO: 23 - DNA, 20 bp, synthetic construct
  source 1..20: mol_type = other DNA
aaactcgtactcgcttctcc

SEQ ID NO: 24 - DNA, 35 bp, synthetic construct
  source 1..35: mol_type = other DNA
atgcctgcaggtcgaccggcgccggcaacctcgtc

SEQ ID NO: 25 - DNA, 33 bp, synthetic construct
  source 1..33: mol_type = other DNA
cggtacccggggatccttcatcgatagggtggg

SEQ ID NO: 26 - DNA, 34 bp, synthetic construct
  source 1..34: mol_type = other DNA
gtactcctcagcttactcatcctttgcatcaaca

SEQ ID NO: 27 - DNA, 34 bp, synthetic construct
  source 1..34: mol_type = other DNA
agtaagctgaggagtactgcctgccaaccatcaa

SEQ ID NO: 28 - DNA, 34 bp, synthetic construct
  source 1..34: mol_type = other DNA
atgcctgcaggtcgaccgactggcttgccaccct

SEQ ID NO: 29 - DNA, 2196 bp, synthetic construct
  source 1..2196: mol_type = other DNA
atgagttcttctcttaaaattgcttcgactcaagaagcgcgtcaatatttcgatactgaccgcgttgttgtcgatgctgtaggctctgattttactgatgtcggtgctgttatcgcaatggattacgaaacagatgtcatcgacgctgctgatgcaactaagtttggtattcctgtttttgccgtaactaaggatgcccaagctatcagtgctgatgagctgaagaagattttccacatcattgatttggaaaacaaatttgatgctactgttaacgctcgtgaaatcgaaactgctgttaacaactacgaagacagcattttaccaccattcttcaagtcattgaaagaatacgttagccgtggtttaatccaattcgactgcccaggtcaccaaggtggtcaatactacagaaagcacccagctggtcgtgaattctacgacttcttcggcgaaactgtcttccgtgcagacttatgtaacgctgacgttgccttgggtgacttgctgatccacgaaggtcctgctgttgctgctgaaaagcatgctgcacgtgtttacaacgctgacaagacttacttcgttttaggtggttcttccaacgctaacaacactgtaacatctgctttagtttctaacggcgacttggtattgttcgaccggaacaaccacaagtccgtttacaactcagctttagctatggctggtggccgtcctgtttacctccaaacaaaccgtaacccatacggcttcatcggtggtatctacgacagcgacttcgatgaaaagaagatccgtgaactggcagctaaggttgacccagaacgtgctaagtggaagcgtccattccgtctggctgttatccaattaggtacttacgatggtactatctacaacgcacacgaagttgtaaagcgtatcggtcacctttgtgattacatcgaattcgactctgcttgggtaggttacgaacaattcattcctatgatgcgtaactcttcaccattattgattgatgaccttggtccagaagatcctggtatcattgttgttcaatcagttcacaagcaacaagccggcttctcacaaacttcacaaatccacaagaaggatagccacatcaagggtcaattacgttactgtgaccacaagcactttaacaactccttcaacttgttcatgtctacttcaccattctacccaatgtatgcagcattagacgttaacgctgctatgcaagaaggcgaagcaggtcgcaagttatggcatgaccttctgattactaccattgaagctcgtaagaagttgatcaaggctggctcaatgttccgtccattcgttccacctgttgttaacggcaagaagtgggaagatggcgacactgaagatatggctaacaacattgactactggcgctttgaaaagggtgctaagtggcatgcttacgaaggctacggcgacaaccaatactacgttgatccaaacaagttcatgttaactacacctggtatcaacccagaaactggtgactacgaagacttcggtgttccagctactatcgttgctaactacttacgtgaccacggtatcatccctgaaaagtctgacttgaactctatcttgttcttgatgactccagctgaaactccagctaagatgaacaacctgatcactcaacttcttcaattacaacgcttgatcgaagaagatgctccattgaagcaagttcttccttcaatctacgctgctaacgaagaacgttacaatggctacactatccgtgaactttgccaagaattgcacgacttctacaagaacaacaacacgttcacataccagaagcgtctcttcttacgtgaattcttcccagaacaaggtatgcttccatacgaagctcgtcaagaattcatccgcaaccacaacaagcttgttccattgaacaagatcgaaggcgaaatcgccctcgaaggtgctcttccataccctccaggagtattctgtgtagcaccaggtgaaaagtggtcagaaactgctgttaagtacttcactatcttacaagatggtatcaacaacttccctggattcgctccagaaatccaaggtgtatacttcaagcaagaaggcgacaaggttgttgcttacggtgaagtttacgatgcagaagttgctaagaacgatgatcgttacaacaactaa

SEQ ID NO: 30 - DNA, 2196 bp, synthetic construct
  source 1..2196: mol_type = other DNA
atgtcctcttcacttaaaattgcctcgacccaagaagctcgtcagtatttcgataccgaccgtgtggttgtagacgcagttggatccgacttcactgatgtgggagcagtaattgccatggactacgagaccgacgtaattgacgctgcagacgcaaccaaatttggaatcccggtattcgctgtaactaaggacgctcaggcaatttcggccgacgagcttaagaagatctttcacattattgacctcgaaaataagttcgatgctacggtaaacgcccgcgaaattgagactgcagtcaataactacgaagattctatccttccccctttttttaagtcccttaaggagtacgtctcacgcggacttattcagttcgactgcccaggccatcaaggtggacagtactatcggaaacatcccgctggtcgcgaattttacgactttttcggtgaaacggtcttccgtgccgacctctgcaacgcggatgttgcccttggtgaccttctcattcatgagggacccgcggtcgccgctgaaaagcacgcggcacgtgtctacaatgccgacaaaacctattttgtcttgggaggaagctcgaacgctaataacactgtaacttccgccctggtgtccaacggcgacttggtgctgttcgatcgtaataaccataaaagcgtgtacaactcggcacttgcaatggcgggaggtcggcccgtatatttgcagactaatcgtaatccttatggttttattggaggcatctatgattcggattttgacgaaaaaaaaatccgtgaattggctgcgaaggtcgatcctgaacgtgctaaatggaagcgtccgttccggctggctgtgattcagctgggaacttacgacggaactatctataacgcacatgaagtggtgaagcgtatcggtcatttgtgcgactatatcgaattcgattcagcctgggtcggctatgaacagtttatccctatgatgcgcaattcctccccgcttcttatcgacgacctgggtccagaagaccccggaatcattgtagtccaatcggttcataagcagcaagcaggtttctcgcagactagccagattcacaaaaaagactcgcatattaaaggacagcttcggtactgtgaccataagcattttaataacagcttcaacttgttcatgtctaccagccctttttaccctatgtacgcagcactcgacgtaaacgcggcaatgcaggaaggagaggcaggtcggaaactctggcacgatctcttgattacgacgatcgaagcccggaaaaaactcatcaaagctggttccatgttccgtccatttgtaccacctgttgtgaatggtaagaaatgggaagatggagatactgaggatatggccaataacattgattactggcgtttcgaaaaaggtgcgaagtggcatgcatatgaaggctacggcgataatcaatattatgtcgacccaaacaagtttatgttgactactcctggaattaatccggagactggtgattacgaagacttcggcgttcctgcaactatcgttgctaattatcttcgtgaccacggcatcattccagaaaaatccgacctgaatagcattctttttctcatgacccccgcggagacgccggcgaaaatgaataacctgattacgcagttgctgcaactccaacggctcattgaggaggatgctccgcttaaacaagtactgccttcaatttatgccgctaacgaagagcggtataatggatacactatccgtgagctgtgccaggagttgcacgatttttacaagaacaacaatacgttcacctaccagaaacgcctcttcttgcgtgaattttttcccgaacagggaatgttgccatatgaggcgcgtcaagaatttattcgcaaccacaacaagttggttcccctgaacaaaattgaaggcgaaattgccctcgagggcgcgctgccttatcctcctggcgtcttctgtgtggctcctggagagaaatggtcagaaacggcagtgaagtattttaccatccttcaggacggcattaataattttccaggattcgcgcccgagatccaaggtgtgtacttcaagcaggagggagacaaagtagtattgtatggtgaagtgtacgatgcagaagttgccaaaaatgacgaccggtataataattaa

SEQ ID NO: 31 - DNA, 37 bp, synthetic construct
  source 1..37: mol_type = other DNA
gaaaggaaacactcatgtcctcttcacttaaaattgc

SEQ ID NO: 32 - DNA, 39 bp, synthetic construct
  source 1..39: mol_type = other DNA
cttaaatcgccttcagggttaattattataccggtcgtc

SEQ ID NO: 33 - DNA, 32 bp, synthetic construct
  source 1..32: mol_type = other DNA
cgctattctggtatccagaaacatcccagcgc

SEQ ID NO: 34 - DNA, 38 bp, synthetic construct
  source 1..38: mol_type = other DNA
ttttaagtgaagaggacatgagtgtttcctttcgttgg

SEQ ID NO: 35 - DNA, 37 bp, synthetic construct
  source 1..37: mol_type = other DNA
agctcggtacccggggatcccaggaatacagctgttc

SEQ ID NO: 36 - DNA, 34 bp, synthetic construct
  source 1..34: mol_type = other DNA
ctgggatgtttctggataccagaatagcgaaatg

SEQ ID NO: 37 - DNA, 39 bp, synthetic construct
  source 1..39: mol_type = other DNA
gacgaccggtataataattaaccctgaaggcgatttaag

SEQ ID NO: 38 - DNA, 34 bp, synthetic construct
  source 1..34: mol_type = other DNA
gcctgcaggtcgactctagaaatggcagagttgg

SEQ ID NO: 39 - DNA, 5930 bp, synthetic construct
  source 1..5930: mol_type = other DNA
cggctggctggtttattgctgataaatctggagccggtgagcgtgggtctcgcggtatcattgcagcactggggccagatggtaagccctcccgtatcgtagttatctacacgacggggagtcaggcaactatggatgaacgaaatagacagatcgctgagataggtgcctcactgattaagcattggtaactgtcagaccaagtttactcatatatactttagattgatttaaaacttcatttttaatttaaaaggatctaggtgaagatcctttttgataatctcatgaccaaaatcccttaacgtgagttttcgttccactgagcgtcagaccccttaataagatgatcttcttgagatcgttttggtctgcgcgtaatctcttgctctgaaaacgaaaaaaccgccttgcagggcggtttttcgaaggttctctgagctaccaactctttgaaccgaggtaactggcttggaggagcgcagtcaccaaaacttgtcctttcagtttagccttaaccggcgcatgacttcaagactaactcctctaaatcaattaccagtggctgctgccagtggtgcttttgcatgtctttccgggttggactcaagacgatagttaccggataaggcgcagcggtcggactgaacggggggttcgtgcatacagtccagcttggagcgaactgcctacccggaactgagtgtcaggcgtggaatgagacaaacgcggccataacagcggaatgacaccggtaaaccgaaaggcaggaacaggagagcgcacgagggagccgccagggggaaacgcctggtatctttatagtcctgtcgggtttcgccaccactgatttgagcgtcagatttcgtgatgcttgtcaggggggcggagcctatggaaaaacggctttgccgcggccctctcacttccctgttaagtatcttcctggcatcttccaggaaatctccgccccgttcgtaagccatttccgctcgccgcagtcgaacgaccgagcgtagcgagtcagtgagcgaggaagcggaatatatcctgtatcacatattctgctgacgcaccggtgcagccttttttctcctgccacatgaagcacttcactgacaccctcatcagtgccaacatagtaagccagtatacactccgctagcgctgaggtctgcctcgtgaagaaggtgttgctgactcataccaggcctgaatcgccccatcatccagccagaaagtgagggagccacggttgatgagagctttgttgtaggtggaccagttggtgattttgaacttttgctttgccacggaacggtctgcgttgtcgggaagatgcgtgatctgatccttcaactcagcaaaagttcgatttattcaacaaagccacgttgtgtctcaaaatctctgatgttacattgcacaagataaaaatatatcatcatgaacaataaaactgtctgcttacataaacagtaatacaaggggtgttatgagccatattcaacgggaaacgtcttgctcgaggccgcgattaaattccaacatggatgctgatttatatgggtataaatgggctcgcgataatgtcgggcaatcaggtgcgacaatctatcgattgtatgggaagcccgatgcgccagagttgtttctgaaacatggcaaaggtagcgttgccaatgatgttacagatgagatggtcagactaaactggctgacggaatttatgcctcttccgaccatcaagcattttatccgtactcctgatgatgcatggttactcaccactgcgatccccgggaaaacagcattccaggtattagaagaatatcctgattcaggtgaaaatattgttgatgcgctggcagtgttcctgcgccggttgcattcgattcctgtttgtaattgtccttttaacagcgatcgcgtatttcgtctcgctcaggcgcaatcacgaatgaataacggtttggttgatgcgagtgattttgatgacgagcgtaatggctggcctgttgaacaagtctggaaagaaatgcataagcttttgccattctcaccggattcagtcgtcactcatggtgatttctcacttgataaccttatttttgacgaggggaaattaataggttgtattgatgttggacgagtcggaatcgcagaccgataccaggatcttgccatcctatggaactgcctcggtgagttttctccttcattacagaaacggctttttcaaaaatatggtattgataatcctgatatgaataaattgcagtttcatttgatgctcgatgagtttttctaatcagaattggttaattggttgtaacactggcagagcattacgctgacttgacgggacggcggctttgttgaataaatcgaacttttgctgagttgaaggatcagatcacgcatcttcccgacaacgcagaccgttccgtggcaaagcaaaagttcaaaatcaccaactggtccacctacaacaaagctctcatcaaccgtggctccctcactttctggctggatgatggggcgattcaggcctggtatgagtcagcaacaccttcttcacgaggcagacctcagcgctcaaagatgcaggggtaaaagctaaccgcatctttaccgacaaggcatccggcagttcaacagatcgggaagggctggatttgctgaggatgaaggtggaggaaggtgatgtcattctggtgaagaagctcgaccgtcttggccgcgacaccgccgacatgatccaactgataaaagagtttgatgctcagggtgtagcggttcggtttattgacgacgggatcagtaccgacggtgatatggggcaaatggtggtcaccgcgcgtaatacgactcactatagggcgaattggagctccaccgcggtggcggccgctctagaactagtggatcccccgggctgcaggaattcgatatcaagcttatcgataccgtcgacctcgagggggggcccggtacccagcttttgttccctttagtgagggttaattgcgcggtcaccatcctgtcggctgtggcacaggctgaacgccggaggatcagtactgcggcgtcgctgatcgccctcgcgacgttgtgcgggtggcttgtccctgagggcgctgcgacagatagctaaaaatctgcgtcaggatcgccgtagagcgcgcgtcgcgtcgattggaggcttcccctttggttgacggtcttcaatcgctctacggcgatcctgacgcttttttgttgcgtaccgtcgatcgttttatttctgtcgatcccgaaaaagtttttgccttttgtaaaaaacttctcggtcgccccgcaaattttcgattccagattttttaaaaaccaagccagaaatacgacacaccgtttgcagataatctgtctttcggaaaaatcaagtgcgatacaaaatttttagcacccctgagctgcgcaaagtcccgcttcgtgaaaattttcgtgccgcgtgattttccgccaaaaactttaacgaacgttcgttataatggtgtcatgaccttcacgacgaagtaccaaaattggcccgaatcatcagctatggatctctctgatgtcgcgctggagtccgacgcgctcgatgctgccgtcgatttaaaaacggtgatcggatttttccgagctctcgatacgacggacgcgccagcatcacgagactgggccagtgccgcgagcgacctagaaactctcgtggcggatcttgaggagctggctgacgagctgcgtgctcggcagcgccaggaggacgcacagtagtggaggatcgaatcagttgcgcctactgcggtggcctgattcctccccggcctgacccgcgaggacggcgcgcaaaatattgctcagatgcgtgtcgtgccgcagccagccgcgagcgcgccaacaaacgccacgccgaggagctggaggcggctaggtcgcaaatggcgctggaagtgcgtcccccgagcgaaattttggccatggtcgtcacagagctggaagcggcagcgagaattatccgcgatcgtggcgcggtgcccgcaggcatgacaaacatcgtaaatgccgcgtttcgtgtggccgtggccgcccaggacgtgtcagcgccgccaccacctgcaccgaatcggcagcagcgtcgcgcgtcgaaaaagcgcacaggcggcaagaagcgataagctgcacgaatacctgaaaaatgttgaacgccccgtgagcggtaactcacagggcgtcggctaacccccagtccaaacctgggagaaagcgctcaaaaatgactctagcggattcacgagacattgacacaccggcctggaaattttccgctgatctgttcgacacccatcccgagctcgcgctgcgatcacgtggctggacgagcgaagaccgccgcgaattcctcgctcacctgggcagagaaaatttccagggcagcaagacccgcgacttcgccagcgcttggatcaaagacccggacacgggagaaacacagccgaagttataccgagttggttcaaaatcgcttgcccggtgccagtatgttgctctgacgcacgcgcagcacgcagccgtgcttgtcctggacattgatgtgccgagccaccaggccggcgggaaaatcgagcacgtaaaccccgaggtctacgcgattttggagcgctgggcacgcctggaaaaagcgccagcttggatcggcgtgaatccactgagcgggaaatgccagctcatctggctcattgatccggtgtatgccgcagcaggcatgagcagcccgaatatgcgcctgctggctgcaacgaccgaggaaatgacccgcgttttcggcgctgaccaggctttttcacataggctgagccggtggccactgcacgtctccgacgatcccaccgcgtaccgctggcatgcccagcacaatcgcgtggatcgcctagctgatcttatggaggttgctcgcatgatctcaggcacagaaaaacctaaaaaacgctatgagcaggagttttctagcggacgggcacgtatcgaagcggcaagaaaagccactgcggaagcaaaagcacttgccacgcttgaagcaagcctgccgagcgccgctgaagcgtctggagagctgatcgacggcgtccgtgtcctctggactgctccagggcgtgccgcccgtgatgagacggcttttcgccacgctttgactgtgggataccagttaaaagcggctggtgagcgcctaaaagacaccaagatcatcgacgcctacgagcgtgcctacaccgtcgctcaggcggtcggagcagacggccgtgagcctgatctgccgccgatgcgtgaccgccagacgatggcgcgacgtgtgcgcggctacgtcgctaaaggccagccagtcgtccctgctcgtcagacagagacgcagagcagccgagggcgaaaagctctggccactatgggaagacgtggcggtaaaaaggccgcagaacgctggaaagacccaaacagtgagtacgcccgagcacagcgagaaaaactagctaagtccagtcaacgacaagctaggaaagctaaaggaaatcgcttgaccattgcaggttggtttatgactgttgagggagagactggctcgtggcgacaatcaatgaagctatgtctgaatttagcgtgtcacgtcagaccgtgaatagagcacttaagtctgcgggcattgaacttccacgaggacgccgtaaagcttcccagtaaatgtgccatctcgtaggcagaaaacggttccccccgtaggggtctctctcttggcctcctttctaggtcgggctgattgctcttgaagctctctaggggggctcacaccataggcagataacggttccccaccggctcacctcgtaagcgcacaaggactgctcccaaagatc

SEQ ID NO: 40 - DNA, 5802 bp, synthetic construct
  source 1..5802: mol_type = other DNA
gttcgcttgctgtccataaaaccgcccagtctagctatcgccatgtaagcccactgcaagctacctgctttctctttgcgcttgcgttttcccttgtccagatagcccagtagctgacattcatccggggtcagcaccgtttctgcggactggctttctacgtgttccgcttcctttagcagcccttgcgccctgagtgcttgcggcagcgtgaagctagcttttatcgccattcgccattcaggctgcgcaactgttgggaagggcgatcggtgcgggcctcttcgctattacgccagctggcgaaagggggatgtgctgcaaggcgattaagttgggtaacgccagggttttcccagtcacgacgttgtaaaacgacggccagtgaattcgagctcggtacccggggatcctctagagtcgacctgcaggcatgcaagcttggcgtaatcatggtcatagctgtttcctgtgtgaaattgttatccgctcacaattccacacaacatacgagccggaagcataaagtgtaaagcctggggtgcctaatgagtgagctaactcacattaattgcgttgcgctcactgcccgctttccagtcgggaaacctgtcgtgccagctgcattaatgaatcggccaacgcgcggggagaggcggtttgcgtattgggcgctcttccgcttcctcgctcactgactcgctgcgctcggtcgttcggctgcggcgagcggtatcagctcactcaaaggcggtaatacggttatccacagaatcaggggataacgcaggaaagaacatgtgagcaaaaggccagcaaaaggccaggaaccgtaaaaaggccgcgttgctggcgtttttccataggctccgcccccctgacgagcatcacaaaaatcgacgctcaagtcagaggtggcgaaacccgacaggactataaagataccaggcgtttccccctggaagctccctcgtgcgctctcctgttccgaccctgccgcttaccggatacctgtccgcctttctcccttcgggaagcgtggcgctttctcaatgctcacgctgtaggtatctcagttcggtgtaggtcgttcgctccaagctgggctgtgtgcacgaaccccccgttcagcccgaccgctgcgccttatccggtaactatcgtcttgagtccaacccggtaagacacgacttatcgccactggcagcagccactggtaacaggattagcagagcgaggtatgtaggcggtgctacagagttcttgaagtggtggcctaactacggctacactagaaggacagtatttggtatctgcgctctgctgaagccagttaccttcggaaaaagagttggtagctcttgatccggcaaacaaaccaccgctggtagcggtggtttttttgtttgcaagcagcagattacgcgcagaaaaaaaggatctcaagaagatcctttgatcttttctacggggtctgacgctcagtggaacgaaaactcacgttaagggattttggtcatgagattatcaaaaaggatcttcacctagatccttttggggtgggcgaagaactccagcatgagatccccgcgctggaggatcatccagccctgatagaaacagaagccactggagcacctcaaaaacaccatcatacactaaatcagtaagttggcagcatcacccgacgcactttgcgccgaataaatacctgtgacggaagatcacttcgcagaataaataaatcctggtgtccctgttgataccgggaagccctgggccaacttttggcgaaaatgagacgttgatcggcacgtaagaggttccaactttcaccataatgaaataagatcactaccgggcgtattttttgagttatcgagattttcaggagctgatagaaacagaagccactggagcacctcaaaaacaccatcatacactaaatcagtaagttggcagcatcacccgacgcactttgcgccgaataaatacctgtgacggaagatcacttcgcagaataaataaatcctggtgtccctgttgataccgggaagccctgggccaacttttggcgaaaatgagacgttgatcggcacgtaagaggttccaactttcaccataatgaaataagatcactaccgggcgtattttttgagttatcgagattttcaggagctctttggcatcgtctctcgcctgtcccctcagttcagtaatttcctgcatttgcctgtttccagtcggtagatattccacaaaacagcagggaagcagcgcttttccgctgcataaccctgcttcggggtcattatagcgattttttcggtatatccatcctttttcgcacgatatacaggattttgccaaagggttcgtgtagactttccttggtgtatccaacggcgtcagccgggcaggataggtgaagtaggcccacccgcgagcgggtgttccttcttcactgtcccttattcgcacctggcggtgctcaacgggaatcctgctctgcgaggctggccggctaccgccggcgtaacagatgagggcaagcggatggctgatgaaaccaagccaaccaggaagggcagcccacctatcaaggtgtactgccttccagacgaacgaagagcgattgaggaaaaggcggcggcggccggcatgagcctgtcggcctacctgctggccgtcggccagggctacaaaatcacgggcgtcgtggactatgagcacgtccgcgagggcgtcccggaaaacgattccgaagcccaacctttcatagaaggcggcggtggaatcgaaatctcgtgatggcaggttgggcgtcgcttggtcggtcatttcgaaaaaggttaggaatacggttagccatttgcctgcttttatatagttcatatgggattcacctttatgttgataagaaataaaagaaaatgccaataggatatcggcattttcttttgcgtttttatttgttaactgttaattgtccttgttcaaggatgctgtctttgacaacagatgttttcttgcctttgatgttcagcaggaagctcggcgcaaacgttgattgtttgtctgcgtagaatcctctgtttgtcatatagcttgtaatcacgacattgtttcctttcgcttgaggtacagcgaagtgtgagtaagtaaaggttacatcgttaggcggatcaagatccatttttaacacaaggccagttttgttcagcggcttgtatgggccagttaaagaattagaaacataaccaagcatgtaaatatcgttagacgtaatgccgtcaatcgtcatttttgatccgcgggagtcagtgaacaggtaccatttgccgttcattttaaagacgttcgcgcgttcaatttcatctgttactgtgttagatgcaatcagcggtttcatcacttttttcagtgtgtaatcatcgtttagctcaatcataccgagagcgccgtttgctaactcagccgtgcgttttttatcgctttgcagaagtttttgactttcttgacggaagaatgatgtgcttttgccatagtatgctttgttaaataaagattcttcgccttggtagccatcttcagttccagtgtttgcttcaaatactaagtatttgtggcctttatcttctacgtagtgaggatctctcagcgtatggttgtcgcctgagctgtagttgccttcatcgatgaactgctgtacattttgatacgtttttccgtcaccgtcaaagattgatttataatcctctacaccgttgatgttcaaagagctgtctgatgctgatacgttaacttgtgcagttgtcagtgtttgtttgccgtaatgtttaccggagaaatcagtgtagaataaacggatttttccgtcagatgtaaatgtggctgaacctgaccattcttgtgtttggtcttttaggatagaatcatttgcatcgaatttgtcgctgtctttaaagacgcggccagcgtttttccagctgtcaatagaagtttcgccgactttttgatagaacatgtaaatcgatgtgtcatccgcatttttaggatctccggctaatgcaaagacgatgtggtagccgtgatagtttgcgacagtgccgtcagcgttttgtaatggccagctgtcccaaacgtccaggccttttgcagaagagatatttttaattgtggacgaatcaaattcagaaacttgatatttttcatttttttgctgttcagggatttgcagcatatcatggcgtgtaatatgggaaatgccgtatgtttccttatatggcttttggttcgtttctttcgcaaacgcttgagttgcgcctcctgccagcagtgcggtagtaaaggttaatactgttgcttgttttgcaaactttttgatgttcatcgttcatgtctccttttttatgtactgtgttagcggtctgcttcttccagccctcctgtttgaagatggcaagttagttacgcacaataaaaaaagacctaaaatatgtaaggggtgacgccaaagtatacactttgccctttacacattttaggtcttgcctgctttatcagtaacaaacccgcgcgatttacttttcgacctcattctattagactctcgtttggattgcaactggtctattttcctcttttgtttgatagaaaatcataaaaggatttgcagactacgggcctaaagaactaaaaaatctatctgtttcttttcattctctgtattttttatagtttctgttgcatgggcataaagttgcctttttaatcacaattcagaaaatatcataatatctcatttcactaaataatagtgaacggcaggtatatgtgatgggttaaaaaggatcaccccagagtcccgctcagaagaactcgtcaagaaggcgatagaaggcgatgcgctgcgaatcgggagcggcgataccgtaaagcacgaggaagcggtcagcccattcgccgccaagctcttcagcaatatcacgggtagccaacgctatgtcctgatagcggtccgccacacccagccggccacagtcgatgaatccagaaaagcggccattttccaccatgatattcggcaagcaggcatcgccatgggtcacgacgagatcctcgccgtcgggcatccgcgccttgagcctggcgaacagttcggctggcgcgagcccctgatgctcttcgtccagatcatcctgatcgacaagaccggcttccatccgagtacgtgctcgctcgatgcgatgtttcgcttggtggtcgaatgggcaggtagccggatcaagcgtatgcagccgccgcattgcatcagccatgatggatactttctcggcaggagcaaggtgagatgacaggagatcctgccccggcacttcgcccaatagcagccagtcccttcccgcttcagtgacaacgtcgagacagctgcgcaaggaacgcccgtcgtggccagccacgatagccgcgctgcctcgtcttggagttcattcagggcaccggacaggtcggtcttgacaaaaagaaccgggcgcccctgcgctgacagccggaacacggcggcatcagagcagccgattgtctgttgtgcccagtcatagccgaatagcctctccacccaagcggccggagaacctgcgtgcaatccatcttgttcaatcatgcgaaacgatcctcatcctgtctcttgatcagatcttgatcccctgcgccatcagatccttggcggcaagaaagccatccagtttactttgcagggcttcccaaccttaccagagggcgccccagctggcaattccg

SEQ ID NO: 41 - DNA, 612 bp, synthetic construct
  source 1..612: mol_type = other DNA
atgagtcccaccgttttgcctgctacacaagctgacttccctaagatcgtcgatgttctggttgaagcattcgccaacgatccagcatttttacgatggatcccgcagccggaccccggttcagcaaagcttcgagcacttttcgaactgcagattgagaagcagtatgcagtggcgggaaatattgatgtcgcgcgtgattctgagggagaaatcgtcggcgtcgcgttatgggatcggccagatggtaatcacagtgccaaagatcaagcagcgatactcccccggctcgtctccattttcgggatcaaggctgcgcaggtggcgtggacggatttgagttcggctcgtttccaccccaaattcccccattggtacctctacaccgtggcaacatctagttctgcccgtggaacgggtgttggcagtgcgcttcttaatcacggaatcgctcgcgcgggtgatgaagctatctatttggaggcgacgtcgactcgtgcggctcaactatataaccgtctgggatttgtgcccttgggttatatcccctcagatgatgatggcactcctgaactggcgatgtggaaaccgccagcgatgccaactgtttaa